European Patent Application EP 4 130 278 A1, published February 8, 2023. Title: Novel L-rhamnose isomerase. Applicant: NATIONAL UNIVERSITY CORPORATION KAGAWA UNIVERSITY. The sequence listing filed with the application follows.

SEQUENCE LISTING (60 sequences)

SEQ ID NO: 1 - protein, 418 aa, Erwinia billingiae
  Inventor: Akimitsu, Kazuya; Izumori, Ken; Yoshihara, Akihide; Kato, Shiro; Mochizuki, Susumu; Yoshida, Hiromi; Kamitori, Shigehiro; Seq-1
MTKLIEQAYELAKQRYADVGIDVEQVMTQLDGIPVSMHCWQGDDVRGFENPNGELTGGIQATGNYPGRARNAHELRADIEKAMSLIPGAKRLNLHAIYLESDTPVERDAIEPQHFSHWVEWAKQHKLGLDFNPSCFSHPLSADGFTLSHADKGIRQFWIDHCKASRRISAHFGEQLGTPSVMNIWVPDGMKDLTIDRLAPRERLASALDEVISEKFDASHHIDAVESKLFGIGAESYTVGSNEFCLGYAASRQTALTLDAGHFHPTEVISDKISTAMLYVPRLLLHVSRPVRWDSDHVVLLDDETQAIATEIARNKLFNKVHIGLDFFDASINRIAAWVIGTRNAKKALLRALLEPSDQLRKLELEGDYTARLALLEEQKSLPWQAVWEAWCLRHDVPADASWLSEVRHYEQQTLRLR

SEQ ID NO: 2 - DNA, 1257 bp, Erwinia billingiae
  Seq-2
atgacaaagctgattgaacaagcttatgaactggctaaacaacgttacgctgacgtaggaattgatgtggagcaggtgatgacgcaattggatgggattcctgtgtcgatgcactgctggcagggggatgacgtgcgcggcttcgaaaaccccaatggcgaactcaccggcgggattcaggccacaggtaactatccgggacgcgcgcgtaatgcgcatgaactgcgcgccgatatcgaaaaagccatgtcgctgattccaggcgctaagcgcctcaatctgcacgccatctatctggaaagcgacacgccggtagaacgtgatgctatcgaaccgcaacacttcagccactgggtggagtgggcaaaacagcataaattagggctcgattttaatccaagctgcttctcgcatcctttaagtgccgatggttttaccctgtcacacgctgacaaaggcatccgccagttctggattgatcactgcaaggccagtcgccgcatctcggcacattttggtgaacaactgggcacgccctcagtgatgaacatctgggttccggacggtatgaaagatctcaccattgatcgcctggcgccgcgtgaacgtttagccagcgcgctggatgaagtgatcagcgaaaaattcgatgccagtcatcatatcgacgccgtcgaaagtaagttattcgggattggtgctgagagttataccgtggggtccaatgagttttgccttggctacgctgccagccgccagaccgcgctgacacttgatgccgggcatttccatcccactgaagtgatctccgacaaaatctccaccgcgatgctgtatgtcccgcgcctgttattgcacgtcagccgtccggtgcgttgggacagcgaccatgtggtgctgctggatgatgaaacccaggccattgccactgaaattgcgcgtaacaagctgttcaacaaagtgcatatcggcctcgacttctttgatgcttccatcaaccgcatcgcggcgtgggtgattggtacccgcaatgccaaaaaggcgttactgcgtgcgctgttggagccgagtgaccaactgcgcaaactggagcttgagggggattacaccgcacgtctggcgctgctggaggagcaaaagtcattgccatggcaggctgtctgggaagcctggtgcttgcgtcacgatgtccctgctgatgccagttggctcagcgaagtccgtcattatgaacaacaaacactgcgtctacgttaa

SEQ ID NO: 3 - protein, 419 aa, Artificial Sequence
  Seq-3
MTKLIEQAYELAKQRYADVGIDVEQVMTQLDGIPVSMHCWQGDDVRGFENPNGELTGGIQATGNYPGRARNAHELRADIEKAMSLIPGAKRLNLHAIYLESDTPVERDAIEPQHFSHWVEWAKQHKLGLDFNPSCFSHPLSADGFTLSHADKGIRQFWIDHCKASRRISAHFGEQLGTPSVMNIWVPDGMKDLTIDRLAPRERLASALDEVISEKFDASHHIDAVESKLFGIGAESYTVGSNEFCLGYAASRQTALTLDAGHFHPTEVISDKISTAMLYVPRLLLHVSRPVRWDSDHVVLLDDETQAIATEIARNKLFNKVHIGLDFFDASINRIAAWVIGTRNAKKALLRALLEPSDQLRKLELEGDYTARLALLEEQKSLPWQAVWEAWCLRHDVPADASWLSEVRHYEQQTLRLRG

SEQ ID NO: 4 - protein, 418 aa, Artificial Sequence
  Seq-4
MTKLIEQAYELAKQRYADVGIDVEQVMTQLDGIPVSMHCWQGDDVRGFENPNGELTGGIQATGNYPGRARNAHELRADIEKAMSLIPGAKRLNLHAIYLESDTPVERDAIEPQHFSHWVEWAKQHKLGLDFNPSCFSHPLSADGFTLSHADKGIRQFWIDHCKASRRISAHFGEQLGTPSVMNIWVPDGMKDLTIDRLAPRERLASALDEVISEKFDASHHIDAVESKLFGIGAESYTVGSNEFCLGYAASRQTALTLDAGHFHPTEVISDKISTAMLYIPRLLLHVSRPVRWDSDHVVLLDDETQAIATEIARNKLFNKVHIGLDFFDASINRIAAWVIGTRNAKKALLRALLEPSDQLRKLELEGDYTARLALLEEQKSLPWQAVWEAWCLRHDVPADASWLSEVRHYEQQTLRLR

SEQ ID NO: 5 - protein, 418 aa, Artificial Sequence
  Seq-5
MTKLIEQAYELAKQRYADVGIDVEQVMTQLDGIPVSMHCWQGDDVRGFENPNGELTGGIQATGNYPGRARNAHELRADIEKAMSLIPGAKRLNLHAIYLESDTPVERDAIEPQHFSHWVEWAKQHKLGLDFNPSCFSHPLSADGFTLSHADKGIRQFWIDHCKASRRISAHFGEQLGTPSVMNIWVPDGMKDLTIDRLAPRERLASALDEVISEKFDASHHIDAVESKLFGIGAESYTVGSNEFCLGYAASRQTALTLDAGHFHPTEVISDKISTAMLYVPRLLLHVSRPVRWDSDHVVLLDDETQAIATEIARNKLFNKVHIGLDFFDASINRIAAWVIGTRNAKKALLRALLEPSDQLRKLELEGDYTARLALLEEQKSLPWQAIWEAWCLRHDVPADASWLSEVRHYEQQTLRLR

SEQ ID NO: 6 - protein, 418 aa, Artificial Sequence
  Seq-6
MTKLIEQAYELAKQRYADVGIDVEQVMTQLDGIPVSMHCWQGDDVRGFENPNGELTGGIQATGNYPGRARNAHELRADIEKAMSLIPGAKRLNLHAIYLESDTPVERDAIEPQHFSHWVEWAKQHKLGLDFNPSCFSHPLSADGFTLSHADKGIRQFWIDHCKASRRISAHFGEQLGTPSVMNIWVPDGMKDLTIDRFAPRERLASALDEVISEKFDASHHIDAVESKLFGIGAESYTVGSNEFCLGYAASRQTALTLDAGHFHPTEVISDKISTAMLYVPRLLLHVSRPVRWDSDHVVLLDDETQAIATEIARNKLFNKVHIGLDFFDASINRIAAWVIGTRNAKKALLRALLEPSDQLRKLELEGDYTARLALLEEQKSLPWQAVWEAWCLRHDVPADASWLSEVRHYEQQTLRLR

SEQ ID NO: 7 - protein, 418 aa, Artificial Sequence
  Seq-7
MTKLIEQAYELAKQRYADVGIDVEQVMTQLDGIPVSMHCWQGDDVRGFENPNGELTGGIQATGNYPGRARNAHELRADIEKAMSLIPGAKRLNLHAIYLESDTPVERDAIEPQHFSHWVEWAKQHKLGLDFNPSCFSHPLSADGFTLSHADKGIRQFWIDHCKASRRISAHFGEQLGTPSVMNIWVPDGMKDLTIDRLAPRERLASALDEVISEKFDASHHIDAVESKLFGIGAESYTVGSNEFCLGYAASRQTALTLDAGHFHPTEVISDKISTAMLYVPRLLLHVSRPVRWDSDHVVLLDDETQAIATEIARNKLFNKVHIGLDFFDASINRIAAWVIGTRNAKKALLRALLEPSDQLRKLELEGDYTARLALLEEQKSLPWQAVWEAWCLRHDVPADASWLEEVRHYEQQTLRLR

SEQ ID NO: 8 - protein, 418 aa, Artificial Sequence
  Seq-8
MTKLIEQAYELAKQRYADVGIDVEQVMTQLDGIPVSMHCWQGDDVRGFENPEGELTGGIQATGNYPGRARNAHELRADIEKAMSLIPGAKRLNLHAIYLESDTPVERDAIEPQHFSHWVEWAKQHKLGLDFNPSCFSHPLSADGFTLSHADKGIRQFWIDHCKASRRISAHFGEQLGTPSVMNIWVPDGMKDLTIDRLAPRERLASALDEVISEKFDASHHIDAVESKLFGIGAESYTVGSNEFCLGYAASRQTALTLDAGHFHPTEVISDKISTAMLYVPRLLLHVSRPVRWDSDHVVLLDDETQAIATEIARNKLFNKVHIGLDFFDASINRIAAWVIGTRNAKKALLRALLEPSDQLRKLELEGDYTARLALLEEQKSLPWQAVWEAWCLRHDVPADASWLSEVRHYEQQTLRLR

SEQ ID NO: 9 - protein, 418 aa, Artificial Sequence
  Seq-9
MTKLIEQAYELAKQRYADVGIDVEQVMTQLDGIPVSMHCWQGDDVRGFENPNGELTGGIQATGNYPGRARNAHELRADIEKAMSLIPGAKRLNLHAIYLESDTPVERDAIEPQHFSHWVEWAKRHKLGLDFNPSCFSHPLSADGFTLSHADKGIRQFWIDHCKASRRISAHFGEQLGTPSVMNIWVPDGMKDLTIDRLAPRERLASALDEVISEKFDASHHIDAVESKLFGIGAESYTVGSNEFCLGYAASRQTALTLDAGHFHPTEVISDKISTAMLYVPRLLLHVSRPVRWDSDHVVLLDDETQAIATEIARNKLFNKVHIGLDFFDASINRIAAWVIGTRNAKKALLRALLEPSDQLRKLELEGDYTARLALLEEQKSLPWQAVWEAWCLRHDVPADASWLSEVRHYEQQTLRLR

SEQ ID NO: 10 - protein, 418 aa, Artificial Sequence
  Seq-10
MTKLIEQAYELAKQRYADVGIDVEQVMTQLDGIPVSMHCWQGDDVRGFENPNGELTGGIQATGNYPGRARNAHELRADIEKAMSLIPGAKRLNLHAIYLESTTPVERDAIEPQHFSHWVEWAKQHKLGLDFNPSCFSHPLSADGFTLSHADKGIRQFWIDHCKASRRISAHFGEQLGTPSVMNIWVPDGMKDLTIDRLAPRERLASALDEVISEKFDASHHIDAVESKLFGIGAESYTVGSNEFCLGYAASRQTALTLDAGHFHPTEVISDKISTAMLYVPRLLLHVSRPVRWDSDHVVLLDDETQAIATEIARNKLFNKVHIGLDFFDASINRIAAWVIGTRNAKKALLRALLEPSDQLRKLELEGDYTARLALLEEQKSLPWQAVWEAWCLRHDVPADASWLSEVRHYEQQTLRLR

SEQ ID NO: 11 - protein, 418 aa, Artificial Sequence
  Seq-11
MTKLIEQAYELAKQRYADVGIDVEQVMTQLDGIPVSMHCWQGDDVRGFENPNGELTGGIQATGNYPGRARNAHELRADIEKAMSLIPGAKRLNLHAIYLESDTPVERDAIEPQHFSHWVEWAKQHKLGLDFNPSCFSHPLSADGFTLSHADKGIRQFWIDHCKASRRISAHFGEQLGTPSVMNIWVPDGMKDLTIDRLAPRERLASALDEVISEKFDASHHIDAVESKLFGIGAESYTVGSNEFCLGYAASRQTALTLDAGHFHPTEVISDKISTAMLYVPRLLLHVSRPVRWDSDHVVLLDDETQAIATEIARNKLFNKVHIGLDFFDASINRIAAWVIGTRNAKKALLRALLEPSDLLRKLELEGDYTARLALLEEQKSLPWQAVWEAWCLRHDVPADASWLSEVRHYEQQTLRLR

SEQ ID NO: 12 - protein, 418 aa, Artificial Sequence
  Seq-12
MTKLIEQAYELAKQRYADVGIDVEQVMTQLDGIPVSMHCWQGDDVRGFENPNGELTGGIQATGNYPGRARNAHELRADIEKAMSLIPGAKRLNLHAIYLESDTPVERDAIEPQHFSHWVEWAKQHKLGLDFNPSCFSHPLSADGFTLSHADPGIRQFWIDHCKASRRISAHFGEQLGTPSVMNIWVPDGMKDLTIDRLAPRERLASALDEVISEKFDASHHIDAVESKLFGIGAESYTVGSNEFCLGYAASRQTALTLDAGHFHPTEVISDKISTAMLYVPRLLLHVSRPVRWDSDHVVLLDDETQAIATEIARNKLFNKVHIGLDFFDASINRIAAWVIGTRNAKKALLRALLEPSDQLRKLELEGDYTARLALLEEQKSLPWQAVWEAWCLRHDVPADASWLSEVRHYEQQTLRLR

SEQ ID NO: 13 - protein, 418 aa, Artificial Sequence
  Seq-13
MTKLIEQAYELAKQRYAAVGIDVEQVMTQLDGIPVSMHCWQGDDVRGFENPNGELTGGIQATGNYPGRARNAHELRADIEKAMSLIPGAKRLNLHAIYLESDTPVERDAIEPQHFSHWVEWAKQHKLGLDFNPSCFSHPLSADGFTLSHADKGIRQFWIDHCKASRRISAHFGEQLGTPSVMNIWVPDGMKDLTIDRLAPRERLASALDEVISEKLDASHHIDAVESKLFGIGAESYTVGSNEFCLGYAASRQTALTLDAGHFHPTEVISDKISTAMLYVPRLLLHVSRPVRWDSDHVVLLDDETQAIASEIARNKLFNKVHIGLDFFDASINRIAAWVIGTRNAKKALLRALLEPSDQLRKLEQEGDYTARLALLEEQKSLPWQAVWEAWCLRHDVPADASWLSEVRHYEQQTLRLR

SEQ ID NO: 14 - protein, 418 aa, Artificial Sequence
  Seq-14
MTKLIEQAYELAKQRYAAVGIDVEQVMTQLDGIPVSMHCWQGDDVRGFENPNGELTGGIQATGNYPGRARNAHELRADIEKAMSLIPGAKRLNLHAIYLESDTPVERDAIEPQHFSHWVEWAKQHKLGLDFNPSCFSHPLSADGFTLSHADKGIRQFWIDHCKASRRISAHFGEQLGTPSVMNIWVPDGMKDLTIDRLAPRERLASALDEVISEKLDASHHIDAVESKLFGIGAESYTVGSNEFCLGYAASRQTALTLDAGHFHPTEVISDKISTAMLYVPRLLLHVSRPVRWDSDHVVLLDDETQAIATEIARNKLFNKVHIGLDFFDASINRIAAWVIGTRNAKKALLRALLEPSDQLRKLEQEGDYTARLALLEEQKSLPWQAVWEAWCLRHDVPADASWLSEVRHYEQQTLRLR

SEQ ID NO: 15 - protein, 418 aa, Artificial Sequence
  Seq-15
MTKLIEQAFELAKQRYAAIGVDVEKVMAQLDGIPVSMHCWQGDDVRGFENPNGELTGGIQATGNYPGRARNADELRSDVEKAMSLIPGAKRLNLHAIYLESDKPVDRDAIEPKHFSNWVEWAKTHKLGLDFNPSCFSHPLSADGFTLSHADKGIRQFWIDHCKASRRISAHFGEQLGTASVMNIWVPDGMKDLTVDRLGPRQRLASALDEVISEKLNPAHHIDAVESKLFGIGAESYTVGSNEFCLGYASSRQTALTLDAGHFHPTEVISDKISTAMLYVPRLLLHVSRPVRWDSDHVVILDDETQAIATEIARHKLFDKVHIGLDFFDASINRIAAWVIGTRNAKKALLRALLEPTDQLRKLESEGDYTGRLAMLEEQKSLPWQAVWEAWCLRHDVPADASWLSEVRHYEQQTLRQR

SEQ ID NO: 16 - protein, 418 aa, Artificial Sequence
  Seq-16
MTKLIEQAFELAKQRYAAIGVDVEQVMAQLDGIPVSMHCWQGDDVRGFENPNGELTGGIQATGNYPGRARNADELRSDVEKAMSLIPGAKRLNLHAIYLESDKPVDRDAIEPKHFSNWVEWAKTHKLGLDFNPSCFSHPLSADGFTLSHADKGIRQFWIDHCKASRRISAHFGEQLGTASVMNIWVPDGMKDLTVDRLAPRQRLASALDEVISEKLNPAHHIDAVESKLFGIGAESYTVGSNEFCLGYASSRQTALTLDAGHFHPTEVISDKISTAMLYVPRLLLHVSRPVRWDSDHVVILDDETQAIATEIARHKLFDKVHIGLDFFDASINRIAAWVIGTRNAKKALLRALLEPTDQLRKLENEGDYTGRLAMLEEQKSLPWQAVWEAWCLRHDVPADASWLSEVRHYEQQTLRQR

SEQ ID NO: 17 - protein, 418 aa, Artificial Sequence
  Seq-17
MTKLIEQAYELAKQRYAAIGVDVEQVMAQLDGIPVSMHCWQGDDVRGFENPNGELTGGIQATGNYPGRARNADELRSDVEKAMSLIPGAKRLNLHAIYLESDKPVDRDAIEPKHFSNWVEWAKTHKLGLDFNPSCFSHPLSADGFTLSHADKGIRQFWIDHCKASRRISAHFGEQLGTASVMNIWVPDGMKDLTVDRLAPRQRLASALDEVISEKLNPAHHIDAVESKLFGIGAESYTVGSNEFCLGYASSRQTALTLDAGHFHPTEVISDKISTAMLYVPRLLLHVSRPVRWDSDHVVILDDETQAIATEIARHKLFDKVHIGLDFFDASINRIAAWVIGTRNAKKALLRALLEPTDQLRKLESEGDYTGRLAMLEEQKSLPWQAVWEAWCLRHDVPADASWLSEVRHYEQQTLRLR

SEQ ID NO: 18 - protein, 418 aa, Artificial Sequence
  Seq-18
MTKLIEQAYELAKQRYAAIGVDVEQVMAQLDGIPVSMHCWQGDDVRGFENPNGELTGGIQATGNYPGRARNAHELRADVEKAMSLIPGAKRLNLHAIYLESDTPVERDAIEPKHFSNWVEWAKPHKLGLDFNPSCFSHPLSADGFTLSHADKGIRQFWIDHCKASRRISAHFGEQLGTPSVMNIWVPDGMKDLTVDRLAPRQRLASALDEVISEKLDPAHHIDAVESKLFGIGAESYTVGSNEFCLGYATSRQTALTLDAGHFHPTEVISDKISTAMLYVPRLLLHVSRPVRWDSDHVVLLDDETQAIASEIARHKLFDKVHIGLDFFDASINRIAAWVIGTRNAKKALLRALLEPTDQLRKLENEGDYTARLALLEEQKSLPWQAVWEAWCLRHDVPADASWLSEVRHYEQQTLRQR

SEQ ID NO: 19 - protein, 418 aa, Artificial Sequence
  Seq-19
MTKLIEQAYELAKQRYAAIGVDVEQVMAQLDGIPVSMHCWQGDDVRGFENPNGELTGGIQATGNYPGRARNADELRADIEKAMSLIPGAKRLNLHAIYLESDKPVERDAIEPKHFSNWVEWAKNNKLGLDFNPSCFSHPLSADGFTLSHADKGIRQFWIDHCKASRRISAHFGEQLGTPSVMNIWVPDGMKDLTIDRLAPRQRLASALDEVISEKLNPQHHIDAVESKLFGIGAESYTVGSNEFCLGYATSRQTALTLDAGHFHPTEVISDKISTAMLYVPRLLLHVSRPVRWDSDHVVLLDDETQAIATEIARHKLFDKVHIGLDFFDASINRIAAWVIGTRNAKKALLRALLEPSDQLRKLENEGDYTARLALLEEQKSLPWQAVWEAWCLRHDVPADASWLSEVRHYEQQTLRLR

SEQ ID NO: 20 - protein, 418 aa, Artificial Sequence
  Seq-20
MTKLIEQAYELAKQRYAAIGVDVEQVMAQLDGIPVSMHCWQGDDVRGFENPNGELTGGIQATGNYPGRARNADELRADIEKAMSLIPGAKRLNLHAIYLESDKPVERDAIEPKHFSNWVEWAKNNKLGLDFNPSCFSHPLSADGFTLSHADKGIRQFWIDHCKASRRISAHFGEQLGTPSVMNIWVPDGMKDLTVDRLAPRQRLASALDEVISEKLNPQHHIDAVESKLFGIGAESYTVGSNEFCLGYATSRQTALTLDAGHFHPTEVISDKISTAMLYVPRLLLHVSRPVRWDSDHVVLLDDETQAIATEIARHKLFDKVHIGLDFFDASINRIAAWVIGTRNAKKALLRALLEPTDQLRKLENEGDYTARLALLEEQKSLPWQAVWEAWCLRHDVPADASWLSEVRHYEQQTLRLR

SEQ ID NO: 21 - protein, 418 aa, Artificial Sequence
  Seq-21
MTKLIEQAFELAKQRYAAIGVDVEQVLGQLDRIPVSMHCWQGDDVRGFENPQGALTGGIQATGNYPGRARNADELRADLEQAMSLIPGAKRLNLHAIYLESDKPVARDEIEPEHFSNWVEWAKNHQLGLDFNPTCFSHPLSADGFTLSHADKGIRQFWIDHCKASRRISAYFGEQLGTPSVMNIWVPDGMKDLTVDRLAPRQRLASALDEIISEKLNPQHHIDAVESKLFGIGAESYTVGSNEFCLGYATSRQTALTLDAGHFHPTEVISDKISAAMLYVPRLLLHVSRPVRWDSDHVVLLDDETQAIANEIARQNLFDRVHIGLDFFDASINRIAAWVIGTRNAKKALLRALLEPTAQLRQLENEGDYTARLALLEEQKSLPWQAVWEAWCLRHDVPADASWLSDVRHYEQQTLRLR

SEQ ID NO: 22 - protein, 418 aa, Artificial Sequence
  Seq-22
MTKLIEQAYELAKQRYAAIGVDVEQVLGQLDRIPVSMHCWQGDDVRGFENPQGALTGGIQATGNYPGRARNADELRADLEQAMSLIPGAKRLNLHAIYLESDKPVARDEIEPEHFSNWVEWAKNHQLGLDFNPTCFSHPLSADGFTLSHADKGIRQFWIDHCKASRRISAYFGEQLGTPSVMNIWVPDGMKDLTVDRLAPRQRLASALDEIISEKLNPQHHIDAVESKLFGIGAESYTVGSNEFCLGYATSRQTALTLDAGHFHPTEVISDKISAAMLYVPRLLLHVSRPVRWDSDHVVLLDDETQAIANEIARQNLFDRVHIGLDFFDASINRIAAWVIGTRNAKKALLRALLEPTAQLRQLENEGDYTARLALLEEQKSLPWQAVWEAWCLRHDVPADASWLSDVRHYEQQTLRLR

SEQ ID NO: 23 - protein, 418 aa, Artificial Sequence
  Seq-23
MTKLIEQAFELAKQRYAAIGVDVEQVMGQLDGIPVSMHCWQGDDVRGFENPQGALTGGIQATGNYPGRARNADELRADLEKAMSLIPGAKRLNLHAIYLESDKPVERDAIEPEHFSNWVEWAKNHKLGLDFNPTCFSHPLSADGFTLSHADKGIRQFWIDHCKASRRISAYFGEQLGTPSVMNIWVPDGMKDLTVDRLAPRQRLASALDEVISEKLNPQHHIDAVESKLFGIGAESYTVGSNEFCLGYATSRQTALTLDAGHFHPTEVISDKISAAMLYVPRLLLHVSRPVRWDSDHVVLLDDETQAIANEIARQKLFDKVHIGLDFFDASINRIAAWVIGTRNAKKALLRALLEPTDQLRQLENEGDYTARLALLEEQKSLPWQAVWEAWCLRHDVPADASWLSDVRHYEQQTLRLR

SEQ ID NO: 24 - protein, 418 aa, Artificial Sequence
  Seq-24
MTKLIEQAFELAKQRYAAIGVDVEQVMAQLDGIPVSMHCWQGDDVRGFENPQGALTGGIQATGNYPGRARNADELRADLEKAMSLIPGAKRLNLHAIYLESDKPVERDAIEPEHFSNWVEWAKNNKLGLDFNPTCFSHPLSADGFTLSHADKGIRQFWIDHCKASRRISAYFGEQLGTPSVMNIWVPDGMKDLTVDRLAPRQRLASALDEIISEKLNPQHHIDAVESKLFGIGAESYTVGSNEFCLGYATSRQTALTLDAGHFHPTEVISDKISTAMLYVPRLLLHVSRPVRWDSDHVVLLDDETQAIANEIARQKLFDKVHIGLDFFDASINRIAAWVIGTRNAKKALLRALLEPTDQLRQLENEGDYTARLALLEEQKSLPWQAVWEAWCLRHDVPADASWLSDVRHYEQQTLRLR

SEQ ID NO: 25 - protein, 418 aa, Artificial Sequence
  Seq-25
MTKLIEQAYELAKQRYAAIGVDVEQVMAQLDGIPVSMHCWQGDDVRGFENPQGALTGGIQATGNYPGRARNADELRADLEKAMSLIPGAKRLNLHAIYLESDKPVERDAIEPEHFSNWVEWAKKHKLGLDFNPTCFSHPLSADGFTLSHADKGIRQFWIDHCKASRRISAYFGEQLGTPSVMNIWVPDGMKDLTVDRLAPRQRLASALDEIISEKLNPQHHIDAVESKLFGIGAESYTVGSNEFCLGYASSRQTALTLDAGHFHPTEVISDKISTAMLYVPRLLLHVSRPVRWDSDHVVLLDDETQAIANEIARQKLFDKVHIGLDFFDASINRIAAWVIGTRNAKKALLRALLEPTDQLRKLENEGDYTARLALLEEQKSLPWQAVWEAWCLRHDVPADASWLSEVRHYEQQTLRLR

SEQ ID NO: 26 - protein, 418 aa, Artificial Sequence
  Seq-26
MTKLIEQAYELAKQRYAAIGVDVEQAMAQLDRIPVSMHCWQGDDVRGFENPQGALTGGIQATGNYPGRARNADELRADLDKAMSLIPGAKRLNLHAIYLESDKPVERDAIEPEHFSNWVEWAKKHKLGLDFNPTCFSHPLSADGFTLSHADKGIRQFWIDHCKASRRISAYFGEQLGTPSVMNIWVPDGMKDLTVDRLAPRQRLVSALDEVISEKLNPQHHIDAVESKLFGIGAESYTVGSNEFCLGYATSRQTALTLDAGHFHPTEVISDKISTAMLYVPRLLLHVSRPVRWDSDHVVLLDDETQAIANEIARQKLFDKVHIGLDFFDASINRIAAWVIGTRNAKKALLRALLEPTDQLRQLENEGDYTARLALLEEQKSLPWQAVWEAWCLRHDVPADASWLSEVRHYEQQTLRLR

SEQ ID NO: 27 - protein, 418 aa, Artificial Sequence
  Seq-27
MTKQIEQAFELAKQRYADIGVDVEQAIRQLDRIPVSMHCWQGDDVRGFENPQGALTGGIQATGNYPGRARNADELRSDIDKAMSLIPGAKRLNLHAIYLESDKPVERDAIEPAHFANWVAWAKEHKLGLDFNPSCFSHPMSADGFTLSHSDKTVRQFWIDHCKASRRISAYFGEQLGTPSVMNIWVPDGMKDITVDRLAPRQRLMSALDEVISEKLNPQHHIDAVESKLFGIGAESYTVGSNEFCLGYAASRQTALCLDAGHFHPTEVISDKISAAMLYVPRLLLHVSRPVRWDSDHVVLLDDETQAIASEIVRHQLFDKVHIGLDFFDASINRIAAWVIGTRNTKKALLRALLEPTDRLRQAENEGDYTARLTLLEEQKSLPWQAVWEAWCLRHDVPADASWLGDVRHYEQQTLRLR

SEQ ID NO: 28 - protein, 418 aa, Artificial Sequence
  Seq-28
MTKLIEQAYELAKQRYADIGVDVEQAIRQLDRIPVSMHCWQGDDVRGFENPQGALTGGIQATGNYPGRARNADELRSDIDKAMSLIPGAKRLNLHAIYLESDKPVERDAIEPAHFANWVAWAKEHKLGLDFNPSCFSHPMSADGFTLSHSDKTVRQFWIDHCKASRRISAYFGEQLGTPSVMNIWVPDGMKDITVDRLAPRQRLMSALDEVISEKLNPQHHIDAVESKLFGIGAESYTVGSNEFCLGYAASRQTALCLDAGHFHPTEVISDKISAAMLYVPRLLLHVSRPVRWDSDHVVLLDDETQAIASEIVRHQLFDKVHIGLDFFDASINRIAAWVIGTRNTKKALLRALLEPTDRLRQAENEGDYTARLTLLEEQKSLPWQAVWEAWCLRHDVPADASWLGDVRHYEQQTLRLR

SEQ ID NO: 29 - protein, 418 aa, Artificial Sequence
  Seq-29
MTKLIEQAYELAKQRYAENGVDVDLVMAQLDEIPVSMHCWQGDDVRGFENPNGQLTGGIQATGNYPGRARNADELRADIEKAISLIPGAMRLNLHAIYLESSQPVERDAIEPKHFSNWVAWAKSNRLGLDFNPTCFSHAKSADGFTLSHADTGIRQFWIDHCKASRHISAYFGEQLGTPSVMNIWVPDGMKDLTIDRFAPRQRLASALDAIISEQLNPQHHIDAVESKLFGIGAESYTVGSNEFCLGYASSRQIALTLDAGHFHPTEVISDKISTAMLYVPRLLLHVSRPVRWDSDHVVLLDDETQAIAHEIARQKLFDKVHIGLDFFDASINRIAAWVIGTRNAKKALLRALLEPSDRLRRLESEGDFTARLALLEEQKSLPWQAVWEAWCLRHDVPADASWLSEVRHYEQQTLRLR

SEQ ID NO: 30 - protein, 419 aa, Artificial Sequence
  Seq-30
MTTQLEQAWDLAKQRFAAVGVDVEEALRQLDRLPVSMHCWQGDDVAGFENPGGSLTGGIQATGNYPGKARNATELRADLELTLSLIPGPKRLNLHAIYLESDEPVARNEIKPEHFKNWVEWAKANKLGLDFNPSCFSHPLSADGFTLAHADDEIRQFWIDHVKASRRVSAYFGEQLGTPSVMNIWIPDGMKDITVDRLAPRQRLLAALDEAISEKLDPAHHIDAVESKLFGIGAESYTVGSNEFYMGYAASRQTALCLDAGHFHPTEVISDKISAAMLYVPRLLLHVSRPVRWDSDHVVLLDDETQAIASEIIRHDLFDRVHIGLDFFDASINRIAAWVIGTRNMKKALLRALLEPTAELKKLEANGDYTARLALLEEQKSLPWQAVWEMYCQRNDAPAGSQWLDNVRAYEEDVLSQRG

SEQ ID NO: 31 - protein, 419 aa, Artificial Sequence
  Seq-31
MTTQLEQAWDLAKQRFAAVGVDVEEALRQLDRLPVSMHCWQGDDVAGFENPGGSLTGGIQATGNYPGKARNATELRADLELTLSLIPGPKRLNLHAIYLESDEPVARNEIKPEHFKHWVEWAKANKLGLDFNPSCFSHPLSADGFTLAHADDEIRQFWIDHVKASRRVSAYFGEQLGTPSVMNIWIPDGMKDITVDRLAPRQRLLAALDEAISEKLDPAHHIDAVESKLFGIGAESYTVGSNEFYMGYATSRQTALCLDAGHFHPTEVISDKISAAMLYVPRLLLHVSRPVRWDSDHVVLLDDETQAIASEIIRHDLFDRVHIGLDFFDASINRIAAWVIGTRNMKKALLRALLEPTAELKKLEANGDYTARLALLEEQKSLPWQAVWEMYCQRNDAPAGSQWLDNVRAYEEDVLSQRG

SEQ ID NO: 32 - protein, 419 aa, Artificial Sequence
  Seq-32
MTTQLEQAWDLAKQRFAAVGVDVEEALRQLDRLPVSMHCWQGDDVAGFENPGGSLTGGIQATGNYPGKARNATELRADLELALSLIPGPKRLNLHAIYLESDEPVARNEIKPGHFTNWVEWAKANKLGLDFNPSCFSHPLSADGFTLAHADDEIRQFWIDHVKASRRVSAYFGEQLGTPSVMNIWIPDGMKDITVDRLAPRQRLLAALDEAISEKLDPAHHIDAVESKLFGIGAESYTVGSNEFYMGYATSRQTALCLDAGHFHPTEVISDKISAAMLYVPRLLLHVSRPVRWDSDHVVLLDDETQAIASEIIRHDLFDRVHIGLDFFDASINRIAAWVIGTRNMKKALLRALLEPTAELKKLEANGDYTARLALLEEQKSLPWQAVWEMYCQRNDAPAGSQWLDNVRAYEKDVLSQRG

SEQ ID NO: 33 - protein, 419 aa, Artificial Sequence
  Seq-33
MTTQLEQAWDLAKQRYAAVGVDVDEALRQLDRLPVSMHCWQGDDVAGFENPGGSLTGGIQATGNYPGKARNATELRADLELALSLIPGPKRLNLHAIYLESDTPVARNEIKPAHFKNWVAWAKANQLGLDFNPSCFSHPLSADGFTLAHANDDIRQFWIDHVKASRRVSAYFGEQLGTPSVMNIWIPDGMKDITVDRLAPRQRLLAALDEAISEKLNPAHHIDAVESKLFGIGAESYTVGSNEFYMGYATSRQTALCLDAGHFHPTEVISDKISAAMLYVPRLLLHVSRPVRWDSDHVVLLDDETQAIANEIIRHDLFDRVHIGLDFFDASINRIAAWVIGTRNMKKALLRALLEPTSALKQLEENGDYTARLVLLEEQKTLPWQAVWEMYCQRNDTPAGSQWLDNVRMYEKDVLSQRG

SEQ ID NO: 34 - protein, 418 aa, Artificial Sequence
  Seq-34
MTKLIEQAYEIAKQRYAAVGVDVEEALRQLDRLPVSMHCWQGDDVAGFENPEGSLTGGIQATGNYPGKARNAGELRADLEQALSLIPGPKRLNLHAIYLESDTPVARNEIKPEHFKNWVEWAKANKLGLDFNPSCFSHPLSADGFTLSHANDEIRQFWIDHCKASRRVSAYFGEQLGTPSVMNIWIPDGMKDITVDRFAPRQRLLNALDEVISEKLDPAHHIDAVESKLFGIGAESYTVGSNEFYMGYATSRQTALCLDAGHFHPTEVISDKISAAMLYIPRLLLHVSRPVRWDSDHVVLLDDETQAIASEIIRHNLFDRVHIGLDFFDASINRIAAWVIGTRNMKKALLRALLEPTEQLRQLEADGDYTARLALLEEQKSLPWQAVWEAWCLRHDVPADASWLSEVRHYEQQTLRLR

SEQ ID NO: 35 - protein, 418 aa, Artificial Sequence
  Seq-35
MTKLIEQAYELAKQRYAAVGVDVEEALRQLDRLPVSMHCWQGDDVAGFENPEGSLTGGIQATGNYPGKARNAGELRADLEQALSLIPGPKRLNLHALYLESDTPVARNEIKPEHFKNWVEWAKTNKLGLDFNPSCFSHPLSADGFTLSHANNEIRQFWIDHCKASRRVSAYFGEQLGTPSVMNIWIPDGMKDITVDRFAPRQRLLNALDEVISEKLDPAHHIDAVESKLFGIGAESYTVGSNEFYMGYATSRQTALCLDAGHFHPTEVISDKISAAMLYIPRLLLHVSRPVRWDSDHVVLLDDETQAIASEIIRHNLFDRVHIGLDFFDASINRIAAWVIGTRNMKKALLRALLEPTEQLRQLEADGDYTARLALLEEQKCLPWQAVWEAWCLRHDVPADASWLSEVRHYEQQTLRLR

SEQ ID NO: 36 - protein, 418 aa, Artificial Sequence
  Seq-36
MTKLIEQAYELAKQRFAAVGVDVEEALRQLDRLPVSMHCWQGDDVAGFENPEGALTGGIQATGNYPGKARNATELRADLEQALSLIPGPKRLNLHAIYLESDTPVARNEIKPEHFKNWVEWAKANKLGLDFNPSCFSHPLSADGFTLSHANDEIRQFWIDHCKASRRVSAYFGEQLGTPSVMNIWIPDGMKDITVDRLAPRQRLLDALDEVISEKLDPAHHIDAVESKLFGIGAESYTVGSNEFYMGYATSRQTALCLDAGHFHPTEVISDKISAAMLYVPRLLLHVSRPVRWDSDHVVLLDDETQAIASEIIRHNLFDRVHIGLDFFDASINRIAAWVIGTRNMKKALLRALLEPTDQLRQLEADGDYTARLALLEEQKSLPWQAVWEAWCLRHDVPADASWLSEVRHYEQQTLRLR

SEQ ID NO: 37 - protein, 418 aa, Artificial Sequence
  Seq-37
MTKLIEQAYELAKQRFAAVGVDVEEALRQLDRLPVSMHCWQGDDVAGFENPEGALTGGIQATGNYPGKARNATELRADLEQALSLIPGPKRLNLHAIYLESDTPVARNEIKPEHFKNWVEWAKANKLGLDFNPSCFSHPLSADGFTLSHANDEIRQFWIDHVKASRRVSAYFGEQLGTPSVMNIWIPDGMKDITVDRLAPRQRLLDALDEVISEKLNPAHHIDAVESKLFGIGAESYTVGSNEFYMGYATSRQTALCLDAGHFHPTEVISDKISAAMLYVPRLLLHVSRPVRWDSDHVVLLDDETQAIASEIIRHNLFDRVHIGLDFFDASINRIAAWVIGTRNMKKALLRALLEPTDQLRQLEADGDYTARLALLEEQKSLPWQAVWEAWCLRHDVPADASWLSEVRHYEQQTLRLR

SEQ ID NO: 38 - protein, 418 aa, Artificial Sequence
  Seq-38
MTKLIEQAYELAKQRFAAVGVDVEEALRQLDRLPVSMHCWQGDDVAGFENPEGALTGGIQATGNYPGKARNATELRADLEQALSLIPGPKRLNLHAIYLESDTPVARNEIKPEHFKNWVEWAKANKLGLDFNPSCFSHPLSADGFTLSHANNEIRQFWIDHCKASRRVSAYFGEQLGTPSVMNIWIPDGMKDITVDRLAPRQRLLAALDEVISEKLDPAHHIDAVESKLFGIGAESYTVGSNEFYMGYATSRQTALCLDAGHFHPTEVISDKISAAMLYVPRLLLHVSRPVRWDSDHVVLLDDETQAIASEIIRHNLFDRVHIGLDFFDASINRIAAWVIGTRNMKKALLRALLEPTEQLRQLEADGDYTARLALLEEQKSLPWQAVWEAWCLRHDVPADASWLSEVRHYEQQTLRLR

SEQ ID NO: 39 - protein, 418 aa, Artificial Sequence
  Seq-39
MTKLIEQAYELAKQRFAAVGVDVEEALRQLDRLPVSMHCWQGDDVAGFENPEGALTGGIQATGNYPGKARNATELRADLEQALSLIPGPKRLNLHAIYLESDTPVARNEIKPEHFKNWVEWAKANKLGLDFNPSCFSHPLSADGFTLSHADNEIRQFWIDHCKASRRVSAYFGEQLGTPSVMNIWIPDGMKDITVDRLAPRQRLLAALDEVISEKLDPAHHIDAVESKLFGIGAESYTVGSNEFYMGYATSRQTALCLDAGHFHPTEVISDKISAAMLYVPRLLLHVSRPVRWDSDHVVLLDDETQAIASEIIRHNLFDRVHIGLDFFDASINRIAAWVIGTRNMKKALLRALLEPTEQLRQLEANGDYTARLALLEEQKSLPWQAVWEAWCLRHDVPADASWLSEVRHYEQQTLRLR

SEQ ID NO: 40 - protein, 418 aa, Artificial Sequence
  Seq-40
MTKLIEQAYELAKQRFAAVGIDVEEALRQLDRLPVSMHCWQGDDVAGFENPEGSLTGGIQATGNYPGKARNATELRADLEQALSLIPGPKRLNLHAIYLESDTPVSRDQIKPEHFKNWVEWAKANQLGLDFNPSCFSHPLSADGFTLSHADNKIRQFWIDHCKASRRVSAYFGEQLGTPSVMNIWIPDGMKDITVDRLAPRQRLLDALDEVISEKLDPAHHIDAVESKLFGIGAESYTVGSNEFYMGYATSRQTALCLDAGHFHPTEVISDKISAAMLYVPRLLLHVSRPVRWDSDHVVLLDDETQAIASEIVRHNLFDRVHIGLDFFDASINRIAAWVIGTRNMKKALLRALLEPTEQLRQLEASGDYTARLALLEEQKSLPWQAVWEAWCLRHDVPADASWLSEVRHYEQQTLRLR

SEQ ID NO: 41 - protein, 418 aa, Artificial Sequence
  Seq-41
MTKLIEQAYELAKQRFAAVGIDVEEALRQLDRLPVSMHCWQGDDVAGFENPEGSLTGGIQATGNYPGKARNATELRADLEQALSLIPGPKRLNLHAIYLESDTPVSRDQIKPEHFKNWVEWAKANQLGLDFNPSCFSHPLSADGFTLSHADNKIRQFWIDHCKASRRVSAYFGEQLGTPSVMNIWIPDGMKDITVDRLAPRQRLLAALDEVISEKLDPAHHIDAVESKLFGIGAESYTVGSNEFYMGYATSRQTALCLDAGHFHPTEVISDKISAAMLYVPRLLLHVSRPVRWDSDHVVLLDDETQAIASEIVRHNLFDRVHIGLDFFDASINRIAAWVIGTRNMKKALLRALLEPTEQLRQLEASGDYTARLALLEEQKSLPWQAVWEAWCLRHDVPADASWLSEVRHYEQQTLRLR

SEQ ID NO: 42 - protein, 418 aa, Artificial Sequence
  Seq-42
MTKLIEQAYELAKQRFAAVGVDVEQALPQLDRLPVSMHCWQGDDVAGFENPQGALTGGIQATGNYPGKARNATELRADLEQAMSLIPGPKRLNLHAIYLESDTPVERNAIKPEHFKNWVEWAKEHKLGLDFNPSCFSHPLSADGFTLSHADNDIRQFWIDHCKASRRISAYFGEQLGTPSVMNIWIPDGMKDITVDRLAPRQRLLAALDEVISEKLDPAHHIDAVESKLFGIGAESYTVGSNEFYMGYATSRQTALCLDAGHFHPTEVISDKISAAMLYVPRLLLHVSRPVRWDSDHVVLLDDETQAIASEIIRHNLFDRVHIGLDFFDASINRIAAWVIGTRNMKKALLRALLEPTDQLRQLEANGDYTARLALLEEQKSLPWQAVWEAWCLRHDVPADASWLSEVRHYEQQTLRLR

SEQ ID NO: 43 - protein, 418 aa, Artificial Sequence
  Seq-43
MTKLIEQAYELAKQRFAAVGIDVEEALRQLDRLPVSMHCWQGDDVSGFENPEGSLTGGIQATGNYPGKARNASELRADLEQAMRLIPGPKRLNLHAIYLESDTPVSRDQIKPEHFKNWVEWAKANQLGLDFNPSCFSHPLSADGFTLSHADNSIRQFWIDHCKASRRVSAYFGEQLGTPSVMNIWIPDGMKDITVDRLAPRQRLLAALDEVISEKLDPAHHIDAVESKLFGIGAESYTVGSNEFYMGYATSRQTALCLDAGHFHPTEVISDKISAAMLYVPQLLLHVSRPVRWDSDHVVLLDDETQAIASEIVRHDLFDRVHIGLDFFDASINRIAAWVIGTRNMKKALLRALLEPTAELRKLEAAGDYTARLALLEEQKSLPWQAVWEAWCLRHDVPADASWLSEVRHYEQQTLRLR

SEQ ID NO: 44 - protein, 418 aa, Artificial Sequence
  Seq-44
MTKLIEQAYELAKQRFAAVGIDVEEALRQLDRLPVSMHCWQGDDVSGFENPEGSLTGGIQATGNYPGKARNASELRADLEQAMRLIPGPKRLNLHAIYLESDTPVSRDQIKPEHFKNWVEWAKANQLGLDFNPSCFSHPLSADGFTLSHADNSIRQFWIDHCKASRRVSAYFGEQLGTPSVMNIWIPDGMKDITVDRLAPRQRLLAALDEVISEKLNPAHHIDAVESKLFGIGAESYTVGSNEFYLGYATSRQTALCLDAGHFHPTEVISDKISAAMLYVPQLLLHVSRPVRWDSDHVVLLDDETQAIASEIVRHDLFDRVHIGLDFFDASINRIAAWVIGTRNMKKALLRALLEPTAELRKLEAAGDYTARLALLEEQKSLPWQAVWEAWCLRHDVPADASWLSEVRHYEQQTLRLR

SEQ ID NO: 45 - protein, 418 aa, Artificial Sequence
  Seq-45
MTKLIEQAYELAKQRFAAVGIDVEEALRQLDRLPVSMHCWQGDDVSGFENPEGSLTGGIQATGNYPGKARNASELRTDLEQAMRLIPGPKRLNLHAIYLESDTPVSRDQIKPEHFKNWVEWAKANQLGLDFNPSCFSHPLSADGFTLSHADNSIRQFWIDHCKASRRVSAYFGEQLGTPSVMNIWIPDGMKDITVDRLAPRQRLLAALDEVISEKLNPAHHIDAVESKLFGIGAESYTVGSNEFYMGYATSRQTALCLDAGHFHPTEVISDKISAAMLYVPQLLLHVSRPVRWDSDHVVLLDDETQAIASEIVRHDLFDRVHIGLDFFDASINRIAAWVIGTRNMKKALLRALLEPTAELRKLEAAGDYTARLALLEEQKSLPWQAVWEAWCLRHDVPADASWLSEVRHYEQQTLRLR

SEQ ID NO: 46 - protein, 418 aa, Artificial Sequence
  Seq-46
MTKLIEQAYELAKQRFAAVGVDVEEALRQLDRLPVSMHCWQGDDVAGFENPGGALTGGIQATGNYPGKARNATELRADLELALSLIPGPKRLNLHAIYLESDEPVARNEIKPEHFKNWVEWAKANKLGLDFNPSCFSHPLSADGFTLSHADDEIRQFWIDHVKASRRVSAYFGEQLGTPSVMNIWIPDGMKDITVDRLAPRQRLLAALDEVISEKLNPAHHIDAVESKLFGIGAESYTVGSNEFYMGYATSRQTALCLDAGHFHPTEVISDKISAAMLYVPRLLLHVSRPVRWDSDHVVLLDDETQAIASEIIRHDLFDRVHIGLDFFDASINRIAAWVIGTRNMKKALLRALLEPTAELRQLEADGDYTARLALLEEQKSLPWQAVWEAWCLRHDVPADASWLSEVRHYEQQTLRLR

SEQ ID NO: 47 - protein, 418 aa, Artificial Sequence
  Seq-47
MTKLIEQAYELAKQRFAAVGVDVEEALRQLDRLPVSMHCWQGDDVAGFENPGGALTGGIQATGNYPGKARNATELRADLELALSLIPGPKRLNLHAIYLESDEPVARNEIKPEHFKNWVEWAKANKLGLDFNPSCFSHPLSADGFTLAHADDEIRQFWIDHVKASRRVSAYFGEQLGTPSVMNIWIPDGMKDITVDRLAPRQRLLAALDEVISEKLNPAHHIDAVESKLFGIGAESYTVGSNEFYMGYATSRQTALCLDAGHFHPTEVISDKISAAMLYVPRLLLHVSRPVRWDSDHVVLLDDETQAIASEIIRHDLFDRVHIGLDFFDASINRIAAWVIGTRNMKKALLRALLEPTAELRQLEADGDYTARLALLEEQKSLPWQAVWEAWCLRHDVPADASWLSEVRHYEQQTLRLR

SEQ ID NO: 48 - protein, 418 aa, Artificial Sequence
  Seq-48
MTKLIEQAYELAKQRFAAVGVDVEEALRQLDRLPVSMHCWQGDDVAGFENPGGALTGGIQATGNYPGKARNATELRADLELALSLIPGPKRLNLHAIYLESDEPVARNEIKPEHFKNWVEWAKANKLGLDFNPSCFSHPLSADGFTLAHADNEIRQFWIDHVKASRRVSAYFGEQLGTPSVMNIWIPDGMKDITVDRLAPRQRLLAALDEVISEKLNPAHHIDAVESKLFGIGAESYTVGSNEFYMGYATSRQTALCLDAGHFHPTEVISDKISAAMLYVPRLLLHVSRPVRWDSDHVVLLDDETQAIASEIIRHDLFDRVHIGLDFFDASINRIAAWVIGTRNMKKALLRALLEPTAELRQLEANGDYTARLALLEEQKSLPWQAVWEAWCLRHDVPADASWLSEVRHYEQQTLRLR

SEQ ID NO: 49 - protein, 418 aa, Artificial Sequence
  Seq-49
MTKLIEQAYDLAKQRFAAVGVDVEEALRQLDRLPVSMHCWQGDDVAGFENPGGSLTGGIQATGNYPGKARNATELRADLELALSLIPGPKRLNLHAIYLESDEPVARNEIKPEHFKNWVEWAKANKLGLDFNPSCFSHPLSADGFTLAHADDEIRQFWIDHVKASRRVSAYFGEQLGTPSVMNIWIPDGMKDITVDRLAPRQRLLAALDEAISEKLNPAHHIDAVESKLFGIGAESYTVGSNEFYMGYATSRQTALCLDAGHFHPTEVISDKISAAMLYVPRLLLHVSRPVRWDSDHVVLLDDETQAIASEIIRHDLFDRVHIGLDFFDASINRIAAWVIGTRNMKKALLRALLEPTAELKQLEANGDYTARLALLEEQKSLPWQAVWEAWCLRHDVPADASWLSEVRHYEQQTLRLR

SEQ ID NO: 50 - protein, 418 aa, Artificial Sequence
  Seq-50
MTKLIEQAYDLAKQRFAAVGVDVEEALRQLDRLPVSMHCWQGDDVAGFENPGGSLTGGIQATGNYPGKARNATELRADLELALSLIPGPKRLNLHAIYLESDEPVARNEIKPEHFKNWVEWAKANKLGLDFNPSCFSHPLSADGFTLAHADDEIRQFWIDHVKASRRVSAYFGEQLGTPSVMNIWIPDGMKDITVDRLAPRQRLLAALDEAISEKLDPAHHIDAVESKLFGIGAESYTVGSNEFYMGYATSRQTALCLDAGHFHPTEVISDKISAAMLYVPRLLLHVSRPVRWDSDHVVLLDDETQAIASEIIRHDLFDRVHIGLDFFDASINRIAAWVIGTRNMKKALLRALLEPTAELKQLEANGDYTARLALLEEQKSLPWQAVWEAWCLRHDVPADASWLSEVRHYEQQTLRLR

SEQ ID NO: 51 - protein, 418 aa, Artificial Sequence
  Seq-51
MTKLIEQAYELAKQRFAAVGVDVEEALRQLDRLPVSMHCWQGDDVAGFENPGGSLTGGIQATGNYPGKARNATELRADLELALSLIPGPKRLNLHAIYLESDEPVARNEIKPEHFKNWVEWAKANKLGLDFNPSCFSHPLSADGFTLAHADNEIRQFWIDHVKASRRVSAYFGEQLGTPSVMNIWIPDGMKDITVDRLAPRQRLLAALDEAISEKLDPAHHIDAVESKLFGIGAESYTVGSNEFYMGYATSRQTALCLDAGHFHPTEVISDKISAAMLYVPRLLLHVSRPVRWDSDHVVLLDDETQAIASEIIRHDLFDRVHIGLDFFDASINRIAAWVIGTRNMKKALLRALLEPTAELKQLEANGDYTARLALLEEQKSLPWQAVWEAWCLRHDVPADASWLSEVRHYEQQTLRLR

SEQ ID NO: 52 - protein, 418 aa, Artificial Sequence
  Seq-52
MTKLIEQAYDLAKQRFAAVGVDVEEALRQLDRLPVSMHCWQGDDVAGFENPGGSLTGGIQATGNYPGKARNATELRADLELALSLIPGPKRLNLHAIYLESDEPVARNEIKPEHFKNWVEWAKANRLGLDFNPSCFSHPLSADGFTLAHANDEIRQFWIDHVKASRRVSAYFGEQLGTPSVMNIWIPDGMKDITVDRLAPRQRLLAALDEAISEKLDPAHHIDAVESKLFGIGAESYTVGSNEFYMGYATSRQTALCLDAGHFHPTEVISDKISAAMLYVPRLLLHVSRPVRWDSDHVVLLDDETQAIASEIIRHDLFDRVHIGLDFFDASINRIAAWVIGTRNMKKALLRALLEPVAALKQLEENGDYTARLALLEEQKSLPWQAVWEAWCLRHDVPADASWLSEVRHYEQQTLRLR

SEQ ID NO: 53 - protein, 418 aa, Artificial Sequence
  Seq-53
MTKLIEQAYELAKQRFAAVGVDVEEALRQLDRLPVSMHCWQGDDVAGFENPGGSLTGGIQATGNYPGKARNATELRADLELALSLIPGPKRLNLHAIYLESDEPVARNEIKPEHFKNWVEWAKANRLGLDFNPSCFSHPLSADGFTLAHANNEIRQFWIDHVKASRRVSAYFGEQLGTPSVMNIWIPDGMKDITVDRLAPRQRLLAALDEAISEKLDPAHHIDAVESKLFGIGAESYTVGSNEFYMGYATSRQTALCLDAGHFHPTEVISDKISAAMLYVPRLLLHVSRPVRWDSDHVVLLDDETQAIASEIIRHDLFDRVHIGLDFFDASINRIAAWVIGTRNMKKALLRALLEPVAALKQLEENGDYTARLALLEEQKSLPWQAVWEAWCLRHDVPADASWLSEVRHYEQQTLRLR

SEQ ID NO: 54 - protein, 418 aa, Artificial Sequence
  Seq-54
MTKLIEQAYDLAKQRYAAVGVDVDEALRQLDRLPVSMHCWQGDDVAGFENPGGSLTGGIQATGNYPGKARNATELRADLELALSLIPGPKRLNLHAIYLESDTPVARNEIKPAHFKNWVAWAKANQLGLDFNPSCFSHPLSADGFTLAHANDDIRQFWIDHVKASRRVSAYFGEQLGTPSVMNIWIPDGMKDITVDRLAPRQRLLAALDEAISEKLNPAHHIDAVESKLFGIGAESYTVGSNEFYMGYATSRQTALCLDAGHFHPTEVISDKISAAMLYVPRLLLHVSRPVRWDSDHVVLLDDETQAIASEIIRHDLFDRVHIGLDFFDASINRIAAWVIGTRNMKKALLRALLEPTSALKQLEENGDYTARLVLLEEQKTLPWQAVWEAWCLRHDVPADASWLSEVRHYEQQTLRLR

SEQ ID NO: 55 - protein, 419 aa, Artificial Sequence
  Seq-55
MTTQLEQAWEIAKQRYAAIGVDAEEALRQLDRLPVSMHCWQGDDVAGFENPEGSLTGGIQATGNYPGKARNAQELRADLEQALSLIPGPKRLNLHAIYLESTTPVARNEIKPEHFKHWVEWAKRHQLGLDFNPSCFSHPLSADGFTLSHANPEIRQFWIDHCKASRRISAYFGEQLGTPSVMNIWVPDGMKDITVDRFAPRQRLLNALDEVISEKLDPAHHIDAVESKLFGIGAESYTVGSNEFYMGYAASRQTALCLDAGHFHPTEVISDKISAAMLYIPRLLLHVSRPVRWDSDHVVLLDDETQAIASEIIRHNLFDRVHIGLDFFDASINRIAAWVIGTRNMKKALLRALLEPTALLRQLENDGDYTARLALLEEQKSLPWQAIWEMYCQRHDTPAGSQWLENVRTYEKDVLSQRG

SEQ ID NO: 56 - protein, 419 aa, Artificial Sequence
  Seq-56
MTTQLEQAWELAKQRYAAIGVDVEEALRQLDRLPVSMHCWQGDDVAGFENPDGSLTGGIQATGNYPGKARNAHELRADLEQALSLIPGPKRLNLHAIYLESDTPVARNEIKPEHFKNWVEWAKPHQLGLDFNPSCFSHPLSADGFTLSHANEEIRQFWIDHCKASRRISAYFGEQLGTPSVMNIWVPDGMKDITVDRLAPRQRLLNALDEVISEKLDPAHHIDAVESKLFGIGAESYTVGSNEFYMGYATSRQTALCLDAGHFHPTEVISDKISAAMLYVPRLLLHVSRPVRWDSDHVVLLDDETQAIASEIIRHNLFDRVHIGLDFFDASINRIAAWVIGTRNMKKALLRALLEPTAQLRQLENDGDYTARLALLEEQKSLPWQAVWEMYCQRHDTPAGSQWLDNVRTYEKDVLSQRG

SEQ ID NO: 57 - protein, 418 aa, Artificial Sequence
  Seq-57
MTTQLEQAWELAKQRYAAIGVDVEEALRQLDRLPVSMHCWQGDDVAGFENPEGTLTGGIQATGNYPGKARNANELRADLEQALSLIPGPKRLNLHAIYLESDTPVARNEIKPEHFKNWVEWAKGHQLGLDFNPSCFSHPLSADGFTLSHANEEIRQFWIDHCKASRRISAYFGEQLGTPSVMNIWVPDGMKDITVDRLAPRQRLLNALDEVISEKLDPAHHIDAVESKLFGIGAESYTVGSNEFYMGYAASRQTALCLDAGHFHPTEVISDKISAAMLYVPRLLLHVSRPVRWDSDHVVLLDDETQAIASEIIRHNLFDRVHIGLDFFDASINRIAAWVIGTRNMKKALLRALLEPTALLRQLENDGDYTARLALLEEQKSLPWQAVWEMYCQRHDTPAGSQWLDNVRTYEKQTLRLR

SEQ ID NO: 58 - protein, 418 aa, Artificial Sequence
  Seq-58
MTKLIEQAWELAKQRYAAIGVDVEEALRQLDRLPVSMHCWQGDDVAGFENPEGTLTGGIQATGNYPGKARNANELRADLEQALSLIPGPKRLNLHAIYLESDTPVARNEIKPEHFKNWVEWAKGHQLGLDFNPSCFSHPLSADGFTLSHANEEIRQFWIDHCKASRRISAYFGEQLGTPSVMNIWVPDGMKDITVDRLAPRQRLLNALDEVISEKLDPAHHIDAVESKLFGIGAESYTVGSNEFYMGYAASRQTALCLDAGHFHPTEVISDKISAAMLYVPRLLLHVSRPVRWDSDHVVLLDDETQAIASEIIRHNLFDRVHIGLDFFDASINRIAAWVIGTRNMKKALLRALLEPTALLRQLENDGDYTARLALLEEQKSLPWQAVWEMYCQRHDTPAGSQWLDNVRTYEKQTLRLR

SEQ ID NO: 59 - protein, 418 aa, Artificial Sequence
  Seq-59
MTKLIEQAWELAKQRYAAIGVDVEEALRQLDRLPVSMHCWQGDDVAGFENPEGTLTGGIQATGNYPGKARNANELRADLEQALSLIPGPKRLNLHAIYLESDTPVARNEIKPEHFKNWVEWAKGHQLGLDFNPSCFSHPLSADGFTLSHANEEIRQFWIDHCKASRRISAYFGEQLGTPSVMNIWVPDGMKDITVDRLAPRQRLLNALDEVISEKLDPAHHIDAVESKLFGIGAESYTVGSNEFYMGYAASRQTALCLDAGHFHPTEVISDKISAAMLYVPRLLLHVSRPVRWDSDHVVLLDDETQAIASEIIRHNLFDRVHIGLDFFDASINRIAAWVIGTRNMKKALLRALLEPTALLRQLENDGDYTARLALLEEQKSLPWQAVWEMYCQRHDTPAGSQWLDNVRTYEQQTLRLR

SEQ ID NO: 60 - protein, 419 aa, Artificial Sequence
  Seq-60
MTTQLEQAWELAKQRFAAVGIDVEEALRQLDRLPVSMHCWQGDDVSGFENPEGSLTGGIQATGNYPGKARNASELRADLEQAMRLIPGPKRLNLHAIYLESDTPVSRDQIKPEHFKNWVEWAKANQLGLDFNPSCFSHPLSADGFTLSHADDSIRQFWIDHCKASRRVSAYFGEQLGTPSVMNIWIPDGMKDITVDRLAPRQRLLAALDEVISEKLNPAHHIDAVESKLFGIGAESYTVGSNEFYMGYATSRQTALCLDAGHFHPTEVISDKISAAMLYVPQLLLHVSRPVRWDSDHVVLLDDETQAIASEIVRHDLFDRVHIGLDFFDASINRIAAWVIGTRNMKKALLRALLEPTAELRKLEAPGDYTARLALLEEQKSLPWQAVWEMYCQRHDTPAGSEWLESVRAYEKEILSRRG